European Patent Application EP 4 245 850 A1, published September 20, 2023. Title: Novel gamma-aminobutyrate permease variant and method of producing L-isoleucine using the same. Applicant: CJ CheilJedang Corporation. The sequence listing filed with the application follows.

SEQUENCE LISTING (25 sequences)

SEQ ID NO: 1 - protein, 463 aa, Unknown
  aroP
MAKSNEGLGTGLRTRHLTMMGLGSAIGAGLFLGTGVGIRAAGPAVLLAYIIAGAIVVLVMQMLGEMAAARPASGSFSRYGEDAFGHWAGFSLGWLYWFMLIMVMGAEMTGAAAIMGAWFGVEPWIPSLVCVVFFAVVNLVAVRGFGEFEYWFAFIKVAVIIAFLIIGIALIFGWLPGSTFVGTSNFIGDHGFMPNGISGVAAGLLAVAFAFGGIEIVTIAAAESDKPREAISLAVRAVIWRISVFYLGSVLVITFLMPYESINGADTAAESPFTQILAMANIPGTVGFMEAIIVLALLSAFNAQIYATSRLVFSMANRQDAPRVFSKLSTSHVPTNAVLLSMFFAFVSVGLQYWNPAGLLDFLLNAVGGCLIVVWAMITLSQLKLRKELQANDEISTVRMWAHPWLGILTLVLLAGLVALMLGDAASRSQVYSVAIVYGFLVLLSFVTVNSPLRGGRTPSDLN

SEQ ID NO: 2 - DNA, 1392 bp, Unknown
  aroP
atggctaaatctaatgaagggctgggaaccggacttcggacccgccacctcacaatgatgggactcggctccgcaattggtgccggactgttcctcggcaccggcgttggtatccgcgcagccggccccgcagtgctcctggcgtacatcatcgccggagccatcgttgtgcttgttatgcaaatgctcggcgagatggctgctgcccgtcccgcctccggatcgttttcacgttacggcgaggatgctttcggccactgggctggtttctccctcggttggttgtactggttcatgctgattatggtgatgggcgccgaaatgactggcgctgctgccatcatgggtgcatggttcggcgtcgaaccgtggattccttcgcttgtctgcgtggtcttcttcgctgtggtgaacctcgtcgcggttcgcggtttcggtgaattcgagtactggttcgcattcattaaggtcgcggtgatcatcgctttcctcatcattggtattgctcttattttcggatggcttcccggatccacctttgttggaacctcaaacttcatcggtgatcacggattcatgcccaatggtatttctggtgttgctgctggtttgctcgcggtggcttttgcctttggtggcattgaaattgtcaccattgcagctgcagagtccgataagccacgtgaagctatttccctggcggtgcgtgccgtgatttggcgtatttcagtcttttacttgggctctgttttggtcatcactttcctcatgccttatgagtcgatcaatggtgccgacaccgctgcggaatcccccttcacccaaatcctggcgatggcaaacatccctggcacggttggtttcatggaagcgatcatcgttctagcactgctttccgctttcaacgcccaaatctatgccacttctcgtttggtattttccatggcgaatcgacaagacgctccgcgagttttcagtaagctcagcaccagccacgtccccaccaatgcggtgctgttgtccatgttcttcgccttcgtttcagttggtttgcagtactggaatccagccggtctgcttgatttcctcctcaacgctgttggcggttgtttgattgtggtgtgggcaatgatcactttgtcacagttgaaactccgcaaagaactgcaagcaaacgatgaaatctccacggttcgcatgtgggcgcacccatggttaggcatcctcaccttggttttgttggcaggactcgttgctctcatgctcggcgacgcagcctcccgcagccaggtttactcagtggcaattgtgtacggattcttggttcttttgtccttcgtcacagttaacagcccattgcgcggaggtcgcaccccttccgacttgaactga

SEQ ID NO: 3 - protein, 463 aa, Unknown
  aroP
MAKSNEGLGTGLRTRHLTMMGLGSAIGAGLFLGTGVGIRAAGPAVLLAYIIAGAIVVLVMQMLGEMAAARPASGSFSRYGEDAFGHWAGFSLGWLYWFMLIMVMGAEMTGAAAIMGAWFGVEPWIPSLVCVVFFAVVNLVAVRGFGEFEYWFAFIKVAVIIAFLIIGIALIFGWLPGSTFVGTSNFIGDHGFMPNGISGVAAGLLAVAFAFTGIEIVTIAAAESDKPREAISLAVRAVIWRISVFYLGSVLVITFLMPYESINGADTAAESPFTQILAMANIPGTVGFMEAIIVLALLSAFNAQIYATSRLVFSMANRQDAPRVFSKLSTSHVPTNAVLLSMFFAFVSVGLQYWNPAGLLDFLLNAVGGCLIVVWAMITLSQLKLRKELQANDEISTVRMWAHPWLGILTLVLLAGLVALMLGDAASRSQVYSVAIVYGFLVLLSFVTVNSPLRGGRTPSDLN

SEQ ID NO: 4 - DNA, 36 bp, Artificial Sequence
  primer
aattcgagctcggtacccttccccctggagtccgca

SEQ ID NO: 5 - DNA, 42 bp, Artificial Sequence
  primer
ataggctcggtcgtttttaggcttgtatcaaccgtaaaccca

SEQ ID NO: 6 - DNA, 42 bp, Artificial Sequence
  primer
tgggtttacggttgatacaagcctaaaaacgaccgagcctat

SEQ ID NO: 7 - DNA, 40 bp, Artificial Sequence
  primer
ccttcattagatttagccatgtgtctcctctaaagattgt

SEQ ID NO: 8 - DNA, 40 bp, Artificial Sequence
  primer
acaatctttagaggagacacatggctaaatctaatgaagg

SEQ ID NO: 9 - DNA, 45 bp, Artificial Sequence
  primer
gtcgactctagaggatcccctcagttcaagtcggaaggggtgcga

SEQ ID NO: 10 - DNA, 1338 bp, Unknown
  hom
atgacctcagcatctgccccaagctttaaccccggcaagggtcccggctcagcagtcggaattgcccttttaggattcggaacagtcggcactgaggtgatgcgtctgatgaccgagtacggtgatgaacttgcgcaccgcattggtggcccactggaggttcgtggcattgctgtttctgatatctcaaagccacgtgaaggcgttgcacctgagctgctcactgaggacgcttttgcactcatcgagcgcgaggatgttgacatcgtcgttgaggttatcggcggcattgagtacccacgtgaggtagttctcgcagctctgaaggccggcaagtctgttgttaccgccaataaggctcttgttgcagctcactctgctgagcttgctgatgcagcggaagccgcaaacgttgacctgtacttcgaggctgctgttgcaggcgcaattccagtggttggcccactgcgtcgctccctggctggcgatcagatccagtctgtgatgggcatcgttaacggcaccaccaacttcatcttggacgccatggattccaccggcgctgactatgcagattctttggctgaggcaactcgtttgggttacgccgaagctgatccaactgcagacgtcgaaggccatgacgccgcatccaaggctgcaattttggcatccatcgctttccacacccgtgttaccgcggatgatgtgtactgcgaaggtatcagcaacatcagcgctgccgacattgaggcagcacagcaggcaggccacaccatcaagttgttggccatctgtgagaagttcaccaacaaggaaggaaagtcggctatttctgctcgcgtgcacccgactctattacctgtgtcccacccactggcgtcggtaaacaagtcctttaatgcaatctttgttgaagcagaagcagctggtcgcctgatgttctacggaaacggtgcaggtggcgcgccaaccgcgtctgctgtgcttggcgacgtcgttggtgccgcacgaaacaaggtgcacggtggccgtgctccaggtgagtccacctacgctaacctgccgatcgctgatttcggtgagaccaccactcgttaccacctcgacatggatgtggaagatcgcgtgggggttttggctgaattggctagcctgttctctgagcaaggaatctccctgcgtacaatccgacaggaagagcgcgatgatgatgcacatctgatcgtggtcacccactctgcgctggaatctgatctttcccgcaccgttgaactgctgaaggctaagcctgttgttaaggcaatcaacagtgtgatccgcctcgaaagggactaa

SEQ ID NO: 11 - DNA, 35 bp, Artificial Sequence
  primer
tcgagctcggtaccccgcttttgcactcatcgagc

SEQ ID NO: 12 - DNA, 23 bp, Artificial Sequence
  primer
cacgatcagatgtgcatcatcat

SEQ ID NO: 13 - DNA, 23 bp, Artificial Sequence
  primer
atgatgatgcacatctgatcgtg

SEQ ID NO: 14 - DNA, 35 bp, Artificial Sequence
  primer
ctctagaggatccccgagcatcttccaaaaccttg

SEQ ID NO: 15 - DNA, 1311 bp, Unknown
  ilvA
atgagtgaaacatacgtgtctgagaaaagtccaggagtgatggctagcggagcggagctgattcgtgccgccgacattcaaacggcgcaggcacgaatttcctccgtcattgcaccaactccattgcagtattgccctcgtctttctgaggaaaccggagcggaaatctaccttaagcgtgaggatctgcaggatgttcgttcctacaagatccgcggtgcgctgaactctggagcgcagctcactcaggagcagcgcgatgcaggtatcgttgccgcatctgcaggtaaccatgcccagggcgtggcctatgtgtgcaagtccttgggcgttcagggacgcatctatgttcctgtgcagactccaaagcaaaagcgtgaccgcatcatggttcacggcggagagtttgtctccttggtggtcactggcaataacttcgacgaagcatcggctgcagcgcatgaagatgcagagcgcaccggcgcaacgctgatcgagcctttcgatgctcgcaacaccgtcatcggtcagggtacagtggctgctgagatcttgtcgcagctgacttccatgggcaagagtgcagatcacgtgatggttccagtcggcggtggcggacttcttgcaggtgtggtcagctacatggctgatatggcacctcgcactgcgatcgttggtatcgaaccagcgggagcagcatccatgcaggctgcattgcacaatggtggaccaatcactttggagactgttgatccctttgtggacggcgcagcagtcaaacgtgtcggagatctcaactacaccatcgtggagaagaaccagggtcgcgtgcacatgatgagcgcgaccgagggcgctgtgtgtactgagatgctcgatctttaccaaaacgaaggcatcatcgcggagcctgctggcgcgctgtctatcgctgggttgaaggaaatgtcctttgcacctggttctgtcgtggtgtgcatcatctctggtggcaacaacgatgtgctgcgttatgcggaaatcgctgagcgctccttggtgcaccgcggtttgaagcactacttcttggtgaacttcccgcaaaagcctggtcagttgcgtcacttcctggaagatatcctgggaccggatgatgacatcgcgctggcagagtacctcaagcgcaacaaccgtgagaccggtactgcgttggtgggtattcacttgagtgaagcatcaggattggattctttgctggaacgtatggaggaatcggcaattgattcccgtcgcctcgagccgggcacccctgagtacgaatacttgacctaa

SEQ ID NO: 16 - DNA, 35 bp, Artificial Sequence
  primer
tcgagctcggtacccatgagtgaaacatacgtgtc

SEQ ID NO: 17 - DNA, 39 bp, Artificial Sequence
  primer
gcgcttgaggtactctgccagcgcgatgtcatcatccgg

SEQ ID NO: 18 - DNA, 39 bp, Artificial Sequence
  primer
ccggatgatgacatcgcgctggcagagtacctcaagcgc

SEQ ID NO: 19 - DNA, 34 bp, Artificial Sequence
  primer
ctctagaggatcccccgtcaccgacacctccaca

SEQ ID NO: 20 - protein, 463 aa, Unknown
  aroP
MAKSNEGLGTGLRTRHLTMMGLGSAIGAGLFLGTGVGIRAAGPAVLLAYIIAGAIVVLVMQMLGEMAAARPASGSFSRYGEDAFGHWAGFSLGWLYWFMLIMVMGAEMTGAAAFMGAWFGVEPWIPSLVCVVFFAVVNLVAVRGFGEFEYWFAFIKVAVIIAFLIIGIALIFGWLPGSTFVGTSNFIGDHGFMPNGISGVAAGLLAVAFAFGGIEIVTIAAAESDKPREAISLAVRAVIWRISVFYLGSVLVITFLMPYESINGADTAAESPFTQILAMANIPGTVGFMEAIIVLALLSAFNAQIYATSRLVFSMANRQDAPRVFSKLSTSHVPTNAVLLSMFFAFVSVGLQYWNPAGLLDFLLNAVGGCLIVVWAMITLSQLKLRKELQANDEISTVRMWAHPWLGILTLVLLAGLVALMLGDAASRSQVYSVAIVYGFLVLLSFVTVNSPLRGGRTPSDLN

SEQ ID NO: 21 - protein, 463 aa, Unknown
  aroP
MAKSNEGLGTGLRTRHLTMMGLGSAIGVGLFLGTGVGIRAAGPAVLLAYIIAGAIVVLVMQMLGEMAAARPASGSFSRYGEDAFGHWAGFSLGWLYWFMLIMVMGAEMTGAAAIMGAWFGVEPWIPSLVCVVFFAVVNLVAVRGFGEFEYWFAFIKVAVIIAFLIIGIALIFGWLPGSTFVGTSNFIGDHGFMPNGISGVAAGLLAVAFAFGGIEIVTIAAAESDKPREAISLAVRAVIWRISVFYLGSVLVITFLMPYESINGADTAAESPFTQILAMANIPGTVGFMEAIIVLALLSAFNAQIYATSRLVFSMANRQDAPRVFSKLSTSHVPTNAVLLSMFFAFVSVGLQYWNPAGLLDFLLNAVGGCLIVVWAMITLSQLKLRKELQANDEISTVRMWAHPWLGILTLVLLAGLVALMLGDAASRSQVYSVAIVYGFLVLLSFVTVNSPLRGGRTPSDLN

SEQ ID NO: 22 - DNA, 1392 bp, Unknown
  aroP
atggctaaatctaatgaagggctgggaaccggacttcggacccgccacctcacaatgatgggactcggctccgcaattggtgccggactgttcctcggcaccggcgttggtatccgcgcagccggccccgcagtgctcctggcgtacatcatcgccggagccatcgttgtgcttgttatgcaaatgctcggcgagatggctgctgcccgtcccgcctccggatcgttttcacgttacggcgaggatgctttcggccactgggctggtttctccctcggttggttgtactggttcatgctgattatggtgatgggcgccgaaatgactggcgctgctgccatcatgggtgcatggttcggcgtcgaaccgtggattccttcgcttgtctgcgtggtcttcttcgctgtggtgaacctcgtcgcggttcgcggtttcggtgaattcgagtactggttcgcattcattaaggtcgcggtgatcatcgctttcctcatcattggtattgctcttattttcggatggcttcccggatccacctttgttggaacctcaaacttcatcggtgatcacggattcatgcccaatggtatttctggtgttgctgctggtttgctcgcggtggcttttgcctttaccggcattgaaattgtcaccattgcagctgcagagtccgataagccacgtgaagctatttccctggcggtgcgtgccgtgatttggcgtatttcagtcttttacttgggctctgttttggtcatcactttcctcatgccttatgagtcgatcaatggtgccgacaccgctgcggaatcccccttcacccaaatcctggcgatggcaaacatccctggcacggttggtttcatggaagcgatcatcgttctagcactgctttccgctttcaacgcccaaatctatgccacttctcgtttggtattttccatggcgaatcgacaagacgctccgcgagttttcagtaagctcagcaccagccacgtccccaccaatgcggtgctgttgtccatgttcttcgccttcgtttcagttggtttgcagtactggaatccagccggtctgcttgatttcctcctcaacgctgttggcggttgtttgattgtggtgtgggcaatgatcactttgtcacagttgaaactccgcaaagaactgcaagcaaacgatgaaatctccacggttcgcatgtgggcgcacccatggttaggcatcctcaccttggttttgttggcaggactcgttgctctcatgctcggcgacgcagcctcccgcagccaggtttactcagtggcaattgtgtacggattcttggttcttttgtccttcgtcacagttaacagcccattgcgcggaggtcgcaccccttccgacttgaactga

SEQ ID NO: 23 - DNA, 1392 bp, Unknown
  aroP
atggctaaatctaatgaagggctgggaaccggacttcggacccgccacctcacaatgatgggactcggctccgcaattggtgccggactgttcctcggcaccggcgttggtatccgcgcagccggccccgcagtgctcctggcgtacatcatcgccggagccatcgttgtgcttgttatgcaaatgctcggcgagatggctgctgcccgtcccgcctccggatcgttttcacgttacggcgaggatgctttcggccactgggctggtttctccctcggttggttgtactggttcatgctgattatggtgatgggcgccgaaatgactggcgctgctgccttcatgggtgcatggttcggcgtcgaaccgtggattccttcgcttgtctgcgtggtcttcttcgctgtggtgaacctcgtcgcggttcgcggtttcggtgaattcgagtactggttcgcattcattaaggtcgcggtgatcatcgctttcctcatcattggtattgctcttattttcggatggcttcccggatccacctttgttggaacctcaaacttcatcggtgatcacggattcatgcccaatggtatttctggtgttgctgctggtttgctcgcggtggcttttgcctttggtggcattgaaattgtcaccattgcagctgcagagtccgataagccacgtgaagctatttccctggcggtgcgtgccgtgatttggcgtatttcagtcttttacttgggctctgttttggtcatcactttcctcatgccttatgagtcgatcaatggtgccgacaccgctgcggaatcccccttcacccaaatcctggcgatggcaaacatccctggcacggttggtttcatggaagcgatcatcgttctagcactgctttccgctttcaacgcccaaatctatgccacttctcgtttggtattttccatggcgaatcgacaagacgctccgcgagttttcagtaagctcagcaccagccacgtccccaccaatgcggtgctgttgtccatgttcttcgccttcgtttcagttggtttgcagtactggaatccagccggtctgcttgatttcctcctcaacgctgttggcggttgtttgattgtggtgtgggcaatgatcactttgtcacagttgaaactccgcaaagaactgcaagcaaacgatgaaatctccacggttcgcatgtgggcgcacccatggttaggcatcctcaccttggttttgttggcaggactcgttgctctcatgctcggcgacgcagcctcccgcagccaggtttactcagtggcaattgtgtacggattcttggttcttttgtccttcgtcacagttaacagcccattgcgcggaggtcgcaccccttccgacttgaactga

SEQ ID NO: 24 - DNA, 1392 bp, Unknown
  aroP
atggctaaatctaatgaagggctgggaaccggacttcggacccgccacctcacaatgatgggactcggctccgcaattggtgttggactgttcctcggcaccggcgttggtatccgcgcagccggccccgcagtgctcctggcgtacatcatcgccggagccatcgttgtgcttgttatgcaaatgctcggcgagatggctgctgcccgtcccgcctccggatcgttttcacgttacggcgaggatgctttcggccactgggctggtttctccctcggttggttgtactggttcatgctgattatggtgatgggcgccgaaatgactggcgctgctgccatcatgggtgcatggttcggcgtcgaaccgtggattccttcgcttgtctgcgtggtcttcttcgctgtggtgaacctcgtcgcggttcgcggtttcggtgaattcgagtactggttcgcattcattaaggtcgcggtgatcatcgctttcctcatcattggtattgctcttattttcggatggcttcccggatccacctttgttggaacctcaaacttcatcggtgatcacggattcatgcccaatggtatttctggtgttgctgctggtttgctcgcggtggcttttgcctttggtggcattgaaattgtcaccattgcagctgcagagtccgataagccacgtgaagctatttccctggcggtgcgtgccgtgatttggcgtatttcagtcttttacttgggctctgttttggtcatcactttcctcatgccttatgagtcgatcaatggtgccgacaccgctgcggaatcccccttcacccaaatcctggcgatggcaaacatccctggcacggttggtttcatggaagcgatcatcgttctagcactgctttccgctttcaacgcccaaatctatgccacttctcgtttggtattttccatggcgaatcgacaagacgctccgcgagttttcagtaagctcagcaccagccacgtccccaccaatgcggtgctgttgtccatgttcttcgccttcgtttcagttggtttgcagtactggaatccagccggtctgcttgatttcctcctcaacgctgttggcggttgtttgattgtggtgtgggcaatgatcactttgtcacagttgaaactccgcaaagaactgcaagcaaacgatgaaatctccacggttcgcatgtgggcgcacccatggttaggcatcctcaccttggttttgttggcaggactcgttgctctcatgctcggcgacgcagcctcccgcagccaggtttactcagtggcaattgtgtacggattcttggttcttttgtccttcgtcacagttaacagcccattgcgcggaggtcgcaccccttccgacttgaactga

SEQ ID NO: 25 - protein, 436 aa, Unknown
  ilvA
MSETYVSEKSPGVMASGAELIRAADIQTAQARISSVIAPTPLQYCPRLSEETGAEIYLKREDLQDVRSYKIRGALNSGAQLTQEQRDAGIVAASAGNHAQGVAYVCKSLGVQGRIYVPVQTPKQKRDRIMVHGGEFVSLVVTGNNFDEASAAAHEDAERTGATLIEPFDARNTVIGQGTVAAEILSQLTSMGKSADHVMVPVGGGGLLAGVVSYMADMAPRTAIVGIEPAGAASMQAALHNGGPITLETVDPFVDGAAVKRVGDLNYTIVEKNQGRVHMMSATEGAVCTEMLDLYQNEGIIAEPAGALSIAGLKEMSFAPGSVVVCIISGGNNDVLRYAEIAERSLVHRGLKHYFLVNFPQKPGQLRHFLEDILGPDDDITLFEYLKRNNRETGTALVGIHLSEASGLDSLLERMEESAIDSRRLEPGTPEYEYLT